European Patent Specification EP 3 990 654 B1, published October 4, 2023. Title: Novel monooxygenases for the manufacture of hydroxylated hydrocarbons. Applicant: Covestro Deutschland AG. The sequence listing filed with the application follows.

SEQUENCE LISTING (4 sequences)

SEQ ID NO: 1 - protein, 771 aa, Rhodococcus ruber
MSASVPASACPVDHAALAGGCPVSTNAAAFDPFGPAYQADPAESLRWSRDEEPVFYSPELGYWVVTRYEDVKAVFRDNLVFSPAIALEKITPVSEEATATLARYDYAMARTLVNEDEPAHMPRRRALMDPFTPKELAHHEAMVRRLTREYVDRFVESGKADLVDEMLWEVPLTVALHFLGVPEEDMATMRKYSIAHTVNTWGRPAPEEQVAVAEAVGRFWQYAGTVLEKMRQDPSGHGWMPYGIRMQQQMPDVVTDSYLHSMMMAGIVAAHETTANASANAFKLLLENRPVWEEICADPSLIPNAVEECLRHSGSVAAWRRVATTDTRIGDVDIPAGAKLLVVNASANHDERHFDRPDEFDIRRPNSSDHLTFGYGSHQCMGKNLARMEMQIFLEELTTRLPHMELVPDQEFTYLPNTSFRGPDHVWVQWDPQANPERTDPAVLQRQHPVTIGEPSTRSVSRTVTVERLDRIVDDVLRVVLRAPAGNALPAWTPGAHIDVDLGALSRQYSLCGAPDAPTYEIAVLLDPESRGGSRYVHEQLRVGGSLRIRGPRNHFALDPDAEHYVFVAGGIGITPVLAMADHARARGWSYELHYCGRNRSGMAYLERVAGHGDRAALHVSAEGTRVDLAALLATPVSGTQIYACGPGRLLAGLEDASRHWPDGALHVEHFTSSLTALDPDVEHAFDLDLRDSGLTVRVEPTQTVLDALRANNIDVPSDCEEGLCGSCEVTVLEGEVDHRDTVLTKAERAANRQMMTCCSRACGDRLTLRL

SEQ ID NO: 2 - DNA, 7672 bp, Artificial Sequence
  Expression construct
tggcgaatgggacgcgccctgtagcggcgcattaagcgcggcgggtgtggtggttacgcgcagcgtgaccgctacacttgccagcgccctagcgcccgctcctttcgctttcttcccttcctttctcgccacgttcgccggctttccccgtcaagctctaaatcgggggctccctttagggttccgatttagtgctttacggcacctcgaccccaaaaaacttgattagggtgatggttcacgtagtgggccatcgccctgatagacggtttttcgccctttgacgttggagtccacgttctttaatagtggactcttgttccaaactggaacaacactcaaccctatctcggtctattcttttgatttataagggattttgccgatttcggcctattggttaaaaaatgagctgatttaacaaaaatttaacgcgaattttaacaaaatattaacgtttacaatttcaggtggcacttttcggggaaatgtgcgcggaacccctatttgtttatttttctaaatacattcaaatatgtatccgctcatgaattaattcttagaaaaactcatcgagcatcaaatgaaactgcaatttattcatatcaggattatcaataccatatttttgaaaaagccgtttctgtaatgaaggagaaaactcaccgaggcagttccataggatggcaagatcctggtatcggtctgcgattccgactcgtccaacatcaatacaacctattaatttcccctcgtcaaaaataaggttatcaagtgagaaatcaccatgagtgacgactgaatccggtgagaatggcaaaagtttatgcatttctttccagacttgttcaacaggccagccattacgctcgtcatcaaaatcactcgcatcaaccaaaccgttattcattcgtgattgcgcctgagcgagacgaaatacgcgatcgctgttaaaaggacaattacaaacaggaatcgaatgcaaccggcgcaggaacactgccagcgcatcaacaatattttcacctgaatcaggatattcttctaatacctggaatgctgttttcccggggatcgcagtggtgagtaaccatgcatcatcaggagtacggataaaatgcttgatggtcggaagaggcataaattccgtcagccagtttagtctgaccatctcatctgtaacatcattggcaacgctacctttgccatgtttcagaaacaactctggcgcatcgggcttcccatacaatcgatagattgtcgcacctgattgcccgacattatcgcgagcccatttatacccatataaatcagcatccatgttggaatttaatcgcggcctagagcaagacgtttcccgttgaatatggctcataacaccccttgtattactgtttatgtaagcagacagttttattgttcatgaccaaaatcccttaacgtgagttttcgttccactgagcgtcagaccccgtagaaaagatcaaaggatcttcttgagatcctttttttctgcgcgtaatctgctgcttgcaaacaaaaaaaccaccgctaccagcggtggtttgtttgccggatcaagagctaccaactctttttccgaaggtaactggcttcagcagagcgcagataccaaatactgtccttctagtgtagccgtagttaggccaccacttcaagaactctgtagcaccgcctacatacctcgctctgctaatcctgttaccagtggctgctgccagtggcgataagtcgtgtcttaccgggttggactcaagacgatagttaccggataaggcgcagcggtcgggctgaacggggggttcgtgcacacagcccagcttggagcgaacgacctacaccgaactgagatacctacagcgtgagctatgagaaagcgccacgcttcccgaagggagaaaggcggacaggtatccggtaagcggcagggtcggaacaggagagcgcacgagggagcttccagggggaaacgcctggtatctttatagtcctgtcgggtttcgccacctctgacttgagcgtcgatttttgtgatgctcgtcaggggggcggagcctatggaaaaacgccagcaacgcggcctttttacggttcctggccttttgctggccttttgctcacatgttctttcctgcgttatcccctgattctgtggataaccgtattaccgcctttgagtgagctgataccgctcgccgcagccgaacgaccgagcgcagcgagtcagtgagcgaggaagcggaagagcgcctgatgcggtattttctccttacgcatctgtgcggtatttcacaccgcatatatggtgcactctcagtacaatctgctctgatgccgcatagttaagccagtatacactccgctatcgctacgtgactgggtcatggctgcgccccgacacccgccaacacccgctgacgcgccctgacgggcttgtctgctcccggcatccgcttacagacaagctgtgaccgtctccgggagctgcatgtgtcagaggttttcaccgtcatcaccgaaacgcgcgaggcagctgcggtaaagctcatcagcgtggtcgtgaagcgattcacagatgtctgcctgttcatccgcgtccagctcgttgagtttctccagaagcgttaatgtctggcttctgataaagcgggccatgttaagggcggttttttcctgtttggtcactgatgcctccgtgtaagggggatttctgttcatgggggtaatgataccgatgaaacgagagaggatgctcacgatacgggttactgatgatgaacatgcccggttactggaacgttgtgagggtaaacaactggcggtatggatgcggcgggaccagagaaaaatcactcagggtcaatgccagcgcttcgttaatacagatgtaggtgttccacagggtagccagcagcatcctgcgatgcagatccggaacataatggtgcagggcgctgacttccgcgtttccagactttacgaaacacggaaaccgaagaccattcatgttgttgctcaggtcgcagacgttttgcagcagcagtcgcttcacgttcgctcgcgtatcggtgattcattctgctaaccagtaaggcaaccccgccagcctagccgggtcctcaacgacaggagcacgatcatgcgcacccgtggggccgccatgccggcgataatggcctgcttctcgccgaaacgtttggtggcgggaccagtgacgaaggcttgagcgagggcgtgcaagattccgaataccgcaagcgacaggccgatcatcgtcgcgctccagcgaaagcggtcctcgccgaaaatgacccagagcgctgccggcacctgtcctacgagttgcatgataaagaagacagtcataagtgcggcgacgatagtcatgccccgcgcccaccggaaggagctgactgggttgaaggctctcaagggcatcggtcgagatcccggtgcctaatgagtgagctaacttacattaattgcgttgcgctcactgcccgctttccagtcgggaaacctgtcgtgccagctgcattaatgaatcggccaacgcgcggggagaggcggtttgcgtattgggcgccagggtggtttttcttttcaccagtgagacgggcaacagctgattgcccttcaccgcctggccctgagagagttgcagcaagcggtccacgctggtttgccccagcaggcgaaaatcctgtttgatggtggttaacggcgggatataacatgagctgtcttcggtatcgtcgtatcccactaccgagatatccgcaccaacgcgcagcccggactcggtaatggcgcgcattgcgcccagcgccatctgatcgttggcaaccagcatcgcagtgggaacgatgccctcattcagcatttgcatggtttgttgaaaaccggacatggcactccagtcgccttcccgttccgctatcggctgaatttgattgcgagtgagatatttatgccagccagccagacgcagacgcgccgagacagaacttaatgggcccgctaacagcgcgatttgctggtgacccaatgcgaccagatgctccacgcccagtcgcgtaccgtcttcatgggagaaaataatactgttgatgggtgtctggtcagagacatcaagaaataacgccggaacattagtgcaggcagcttccacagcaatggcatcctggtcatccagcggatagttaatgatcagcccactgacgcgttgcgcgagaagattgtgcaccgccgctttacaggcttcgacgccgcttcgttctaccatcgacaccaccacgctggcacccagttgatcggcgcgagatttaatcgccgcgacaatttgcgacggcgcgtgcagggccagactggaggtggcaacgccaatcagcaacgactgtttgcccgccagttgttgtgccacgcggttgggaatgtaattcagctccgccatcgccgcttccactttttcccgcgttttcgcagaaacgtggctggcctggttcaccacgcgggaaacggtctgataagagacaccggcatactctgcgacatcgtataacgttactggtttcacattcaccaccctgaattgactctcttccgggcgctatcatgccataccgcgaaaggttttgcgccattcgatggtgtccgggatctcgacgctctcccttatgcgactcctgcattaggaagcagcccagtagtaggttgaggccgttgagcaccgccgccgcaaggaatggtgcatgcaaggagatggcgcccaacagtcccccggccacggggcctgccaccatacccacgccgaaacaagcgctcatgagcccgaagtggcgagcccgatcttccccatcggtgatgtcggcgatataggcgccagcaaccgcacctgtggcgccggtgatgccggccacgatgcgtccggcgtagaggatcgagatctcgatcccgcgaaattaatacgactcactataggggaattgtgagcggataacaattcccctctagaaataattttgtttaactttaagaaggagatataccatgggcagcagccatcatcatcatcatcacagcagcggcctggtgccgcgcggcagccatatggctagcatgactggtggacagcaaatgggtcgcggatccgaattcatgagtgcatcagttccggcgtcggcgtgtcccgtcgatcacgcggccctggccggcggctgtccggtgtcgacgaacgccgcggcgttcgatccgttcgggcccgcgtaccaggccgatccggccgagtcgctgcgctggtcccgcgacgaggagccggtgttctacagccccgaactcggctactgggtggtcacccgctacgaggatgtgaaggcggtgttccgcgacaacctcgtgttctcaccggccatcgccctcgagaagatcaccccggtctccgaggaggccaccgccaccctcgcccgctacgactacgccatggcccggaccctcgtgaacgaggacgagcccgcccacatgccgcgccgccgcgcactcatggacccgttcaccccgaaggaactggcgcaccacgaggcgatggtgcgacggctcacgcgcgaatacgtcgaccgcttcgtcgaatccggcaaggccgacctggtggacgagatgctgtgggaggtaccgctcaccgtcgccctgcacttcctcggcgtgccggaggaggacatggcgacgatgcgcaagtactcgatcgcccacaccgtgaacacctggggccgccccgcgcccgaggagcaggtcgccgtcgccgaggcggtcggcaggttctggcagtacgcgggcacggtgctcgagaagatgcgccaggacccctcggggcacggctggatgccctacgggatccgcatgcagcagcagatgccggacgtcgtcaccgactcctacctgcactcgatgatgatggccggcatcgtcgccgcgcacgagaccacggccaacgcgtccgcgaacgcgttcaagctgctgctcgagaaccgcccggtgtgggaggagatctgcgcggatccgtcgctgatccccaacgccgtcgaggagtgcctgcgccactcgggatcggtcgcggcgtggcgacgggtggccaccaccgacacccgcatcggcgacgtcgacatccccgccggcgcaaagctgctcgtcgtcaacgcctccgccaaccatgacgagcggcacttcgaccgtcccgacgagttcgacatccggcgcccgaactcgagcgaccacctcaccttcgggtacggcagccatcagtgcatgggcaagaacctggcccgcatggagatgcagatcttcctcgaggaactgaccacgcggcttccccacatggaactcgtacccgatcaggagttcacctacctgccgaacacctcgttccgcggtcccgatcacgtgtgggtgcagtgggatccgcaggcgaaccccgagcgcaccgacccggccgtgctgcaacggcagcatcccgtcaccatcggcgagccctccacccggtcggtgtcacgcaccgtcaccgtcgagcgcctggaccggatcgtcgacgacgtgctgcgcgtcgtcctacgggctcctgcaggaaatgcgttgcccgcgtggactcctggcgcccacatcgatgtcgacctcggtgcgctgtcgcggcagtactccctgtgcggtgcgcccgacgcgcccacctacgagatcgccgttctgctggaccccgagagccgcggtggctcgcgctacgtccacgaacagctccgggtggggggatcgctccggattcgcgggccccggaaccacttcgcgctcgaccccgacgccgagcactacgtgttcgtggccggcggcatcggcatcacccccgtcctggccatggccgaccacgcccgcgcccgggggtggagctacgaactgcactactgcggccggaaccgttccgggatggcctatctcgagcgggtcgccgggcacggggaccgcgccgccctgcacgtctcggcggaaggcacccgggtcgacctcgccgccctcctcgcgacgccggtgtccggcacccagatctacgcgtgcgggcccggacggctgctcgccggactcgaggacgcgagccggcactggcccgacggtgcgctgcacgtcgagcacttcacctcgtccctcacggcactcgacccggacgtcgagcacgccttcgacctcgacctgcgcgactcgggactcaccgtgcgggtcgagcccacccagaccgtcctcgacgcgttgcgcgccaacaacatcgacgtgcccagcgactgcgaggaaggcctctgcggctcctgcgaggtcaccgtcctcgaaggcgaggtcgaccaccgcgacaccgtgctcaccaaggccgagcgggcggcgaaccggcagatgatgacctgctgctcgcgtgcctgcggcgaccgactgaccctccgactctgaaagcttgcggccgcactcgagcaccaccaccaccaccactgagatccggctgctaacaaagcccgaaaggaagctgagttggctgctgccaccgctgagcaataactagcataaccccttggggcctctaaacgggtcttgaggggttttttgctgaaaggaggaactatatccggat

SEQ ID NO: 3 - DNA, 31 bp, Artificial Sequence
  PCR primer
ctggaattcatgagtgcatcagttccggcgt

SEQ ID NO: 4 - DNA, 27 bp, Artificial Sequence
  PCR primer
catcaagctttcagagtcgcagggcca